European Patent Specification EP 3 423 158 B1, published November 15, 2023. Title: EMBRYONIC CELL-BASED THERAPEUTIC CANDIDATE SCREENING SYSTEMS, MODELS FOR HUNTINGTON'S DISEASE AND USES THEREOF. Applicant: THE ROCKEFELLER UNIVERSITY. The sequence listing filed with the application follows.

SEQUENCE LISTING (70 sequences)

SEQ ID NO: 1 - DNA, 450 bp, Homo sapiens
cagcaacagcagcaacagcagcagcaacagcagcaacagcagcagcagcagcagcagcagcagcagcagcaacaacagcagcagcagcagcaacagcagcagcaacagcagcagcagcagcaacagcagcagcagcaacagcagcagcagcaacagcagcagcagcagcaacagcagcagcagcagcagcagcagcaacagcaacagcagcagcaacagcagcagcagcagcaacagcaacagcagcagcagcagcagcagcaacaacagcagcagcagcagcagcagcaacagcagcaacagcagcaacagcagcaacagcaacagcagcagcagcagcagcagcaacagcagcagcagcaacagcaacagcaacagcaacagcaacagcaacagcagcagcagcagcagcagcagcagcagcagcagcagcaacagcagcagcaacag

SEQ ID NO: 2 - DNA, 7964 bp, Homo sapiens
gtattaccgcctttgagtgagctgataccgctcgccgcagccgaacgaccgagcgcagcgagtcagtgagcgaggaagcggaagagcgcccaatacgcaaaccgcctctccccgcgcgttggccgattcattaatgcagctggcacgacaggtttcccgactggaaagcgggcagtgagcgcaacgcaattaatgtgagttagctcactcattaggcaccccaggctttacactttatgcttccggctcgtatgttgtgtggaattgtgagcggataacaatttcacacaggaaacagctatgaccatgattacgccaagcgcgcaattaaccctcactaaagggaacaaaagctggaggggtcacacttggggtcctcaggtcgtgccgaccacgcgcattctctgcgctctgcgcaggagctcgcccaccctctccccgtgcagagagccccgcagctggctccccgcagggctgtccgggtgagtatggctctggccacgggccagtgtggcgggagggcaaaccccaaggccacctcggctcagagtccacggccggctgtcgccccgctccaggcgtcggcgggggatcctttccgcatgggcctgcgcccgcgctcggcgccccctccacggccccgccccgtccatggccccgtccttcatgggcgagcccctccatggccctgcccctccgcgccccacccctccctcgccccacctctcaccttcctgccccgcccccagcctccccacccctcaccggccagtcccctcccctatcccgctccgcccctcagccgccccgcccctcagccggcctgcctaatgtccccgtccccagcatcgccccgccccgcccccgtctcgccccgcccctcaggcggcctccctgctgtgccccgccccggcctcgccacgcccctacctcaccacgccccccgcatcgccacgccccccgcatcgccacgcctcccttaccatgcagtcccgccccgtcccttcctcgtcccgcctcgccgcgacacttcacacacagcttcgcctcaccccattacagtctcaccacgccccgtcccctctccgttgagccccgcgccttcgcccgggtggggcgctgcgctgtcagcggccttgctgtgtgaggcagaacctgcgggggcaggggcgggctggttccctggccagccattggcagagtccgcaggctagggctgtcaatcatgctggccggcgtggccccgcctccgccggcgcggccccgcctccgccggcgcagcgtctgggacgcaaggcgccgtgggggctgccgggacgggtccaagatggacggccgctcaggttctgcttttaaccctagaaagatagtctgcgtaaaattgacgcatgcattcttgaaatattgctctctctttctaaatagcgcgaatccgtcgctgtgcatttaggacatctcagtcgccgcttggagctcccgtgaggcgtgcttgtcaatgcggtaagtgtcactgattttgaactataacaaccgcgtgagtcaaaatgacgcatgattatcttttacgtgacttttaagatttaactcatacgataattatattgttatttcgtgttctacttacgtgataacttattatatatatattttcttgttatagatatccttctcgagaagcttgatatcgaattccacggggttggggttgcgccttttccaaggcagccctgggtttgcgcagggacgcggctgctctgggcgtggttccgggaaacgcagcggcgccgaccctgggtctcgcacattcttcacgtccgttcgcagcgtcacccggatcttcgccgctacccttgtgggccccccggcgacgcttcctgctccgcccctaagtcgggaaggttccttgcggttcgcggcgtgccggacgtgacaaacggaagccgcacgtctcactagtaccctcgcagacggacagcgccagggagcaatggcagcgcgccgaccgcgatgggctgtggccaatagcggctgctcagcagggcgcgccgagagcagcggccgggaaggggcggtgcgggaggcggggtgtggggcggtagtgtgggccctgttcctgcccgcgcggtgttccgcattctgcaagcctccggagcgcacgtcggcagtcggccccctcgttgaccgaatcaccgacctctctccccagggggatctcgccaccatggggaccgagtacaagcccacggtgcgcctcgccacccgcgacgacgtcccccgggccgtacgcaccctcgccgccgcgttcgccgactaccccgccacgcgccacaccgtcgacccggaccgccacatcgagcgggtcaccgagctgcaagaactcttcctcacgcgcgtcgggctcgacatcggcaaggtgtgggtcgcggacgacggcgccgcggtggcggtctggaccacgccggagagcgtcgaagcgggggcggtgttcgccgagatcggcccgcgcatggccgagttgagcggttcccggctggccgcgcagcaacagatggaaggcctcctggcgccgcaccggcccaaggagcccgcgtggttcctggccaccgtcggcgtctcgcccgaccaccagggcaagggtctgggcagcgccgtcgtgctccccggagtggaggcggccgagcgcgccggggtgcccgccttcctggagacctccgcgccccgcaacctccccttctacgagcggctcggcttcaccgtcaccgccgacgtcgaggtgcccgaaggaccgcgcacctggtgcatgacccgcaagcccggtgccggatccatgcccacgctactgcgggtttatatagacggtcctcacgggatggggaaaaccaccaccacgcaactgctggtggccctgggttcgcgcgacgatatcgtctacgtacccgagccgatgacttactggcaggtgctgggggcttccgagacaatcgcgaacatctacaccacacaacaccgcctcgaccagggtgagatatcggccggggacgcggcggtggtaatgacaagcgcccagataacaatgggcatgccttatgccgtgaccgacgccgttctggctcctcatatcgggggggaggctgggagctcacatgccccgcccccggccctcaccctcatcttcgaccgccatcccatcgccgccctcctgtgctacccggccgcgcgataccttatgggcagcatgaccccccaggccgtgctggcgttcgtggccctcatcccgccgaccttgcccggcacaaacatcgtgttgggggcccttccggaggacagacacatcgaccgcctggccaaacgccagcgccccggcgagcggcttgacctggctatgctggccgcgattcgccgcgtttacgggctgcttgccaatacggtgcggtatctgcagggcggcgggtcgtggcgggaggattggggacagctttcggggacggccgtgccgccccagggtgccgagccccagagcaacgcgggcccacgaccccatatcggggacacgttatttaccctgtttcgggcccccgagttgctggcccccaacggcgacctgtacaacgtgtttgcctgggccttggacgtcttggccaaacgcctccgtcccatgcacgtctttatcctggattacgaccaatcgcccgccggctgccgggacgccctgctgcaacttacctccgggatggtccagacccacgtcaccacccccggctccataccgacgatctgcgacctggcgcgcacgtttgcccgggagatgggggaggctaactgagcggccgcgactctagatcataatcagccataccacatttgtagaggttttacttgctttaaaaaacctcccacacctccccctgaacctgaaacataaaatgaatgcaattgttgttgttaacttgtttattgcagcttataatggttacaaataaagcaatagcatcacaaatttcacaaataaagcatttttttcactgcattctagttgtggtttgtccaaactcatcaatgtatcttaaggaattcgataaaagttttgttactttatagaagaaattttgagtttttgtttttttttaataaataaataaacataaataaattgtttgttgaatttattattagtatgtaagtgtaaatataataaaacttaatatctattcaaattaataaataaacctcgatatacagaccgataaaacacatgcgtcaattttacgcatgattatctttaacgtacgtcacaatatgattatctttctagggttaacctgcggcccagagccccattcattgccccggtgctgagcggcgccgcgagtcggcccgaggcctccggggactgccgtgccgggcgggagaccgccatggcgaccctggaaaagctgatgaaggccttcgagtccctcaagtccttccagcagcagcagcagcagcagcagcagcagcagcagcagcagcagcagcagcagcagcagcagcagcagcagcagcagcagcagcagcagcagcagcagcagcagcagcagcagcagcagcagcagcagcagcagcagcagcagcaacagccgccaccgccgccgccgccgccgccgcctcctcagcttcctcagccgccgccgcaggcacagccgctgctgcctcagccgcagccgcccccgccgccgcccccgccgccacccggcccggctgtggctgaggagccgctgcaccgaccgtgagtttgggcccgctgcagctccctgtcccggcgggtcccaggctacggcggggatggcggtaaccctgcagcctgcgggccggcgacacgaacccccggccccgcagagacagagtgacccagcaacccagagcccatgagggacacccgccccctcctggggcgaggccttcccccacttcagccccgctccctcacttgggtcttcccttgtcctctcgcgaggggaggcagagccttgttggggcctgtcctgaattcaccgaggggagtcacggcctcagccctctcgcccttcgcaggatgcgaagagttggggcgagaacttgtttctttttatttgcgagaaaccagggcgggggttcttttaactgcgttgtgaagagaacttggaggagccgagatttgctcagtgccacttccctcttctagtctgagagggaagagggctgggggcgcgggacacttcgagaggaggcggggtttggagctggagagatgtgggggcagtggatgacataatgcttttaggacgcctcggcgggagtggcggggcagggggggggcggggagtgagggcgcgtccaatgggagatttcttttcctagtggcacttaaaacagcctgagatttgaggctcttcctacattgtcaggacatttcatttagttcatgatcacggtggtagtaacacgattttaagcaccacctaagagatctgctcatctaagcctaagttggtctgcaggcgtttgaatgagttgtggttgccaagtaaagtggtgaacttacgtggtgattaatgaaattatcttaaatattaggaagagttgattgaagttttttgcctatgtgtgttgggaataaaaccaacacgttgctgatggggaggccaattcgccctatagtgagtcgtattacgcgcgctcactggccgtcgttttacaacgtcgtgactgggaaaaccctggcgttacccaacttaatcgccttgcagcacatccccctttcgccagctggcgtaatagcgaagaggcccgcaccgatcgcccttcccaacagttgcgcagcctgaatggcgaatggcgcctgatgcggtattttctccttacgcatctgtgcggtatttcacaccgcatatggtgcactctcagtacaatctgctctgatgccgcatagttaagccagccccgacacccgccaacacccgctgacgcgccctgacgggcttgtctgctcccggcatccgcttacagacaagctgtgaccgtctccgggagctgcatgtgtcagaggttttcaccgtcatcaccgaaacgcgcgagacgaaagggcctcgtgatacgcctatttttataggttaatgtcatgataataatggtttcttagacgtcaggtggcacttttcggggaaatgtgcgcggaacccctatttgtttatttttctaaatacattcaaatatgtatccgctcatgagacaataaccctgataaatgcttcaataatattgaaaaaggaagagtatgagccatattcaacgggaaacgtcttgctctaggccgcgattaaattccaacatggatgctgatttatatgggtataaatgggctcgcgataatgtcgggcaatcaggtgcgacaatctatcgattgtatgggaagcccgatgcgccagagttgtttctgaaacatggcaaaggtagcgttgccaatgatgttacagatgagatggtcagactaaactggctgacggaatttatgcctcttccgaccatcaagcattttatccgtactcctgatgatgcatggttactcaccactgcgatccctgggaaaacagcattccaggtattagaagaatatcctgattcaggtgaaaatattgttgatgcgctggcagtgttcctgcgccggttgcattcgattcctgtttgtaattgtccttttaacagcgatcgcgtatttcgtctcgctcaggcgcaatcacgaatgaataacggtttggttgatgcgagtgattttgatgacgagcgtaatggctggcctgttgaacaagtctggaaagaaatgcataaacttttgccattctcaccggattcagtcgtcactcatggtgatttctcacttgataaccttatttttgacgaggggaaattaataggttgtattgatgttggacgagtcggaatcgcagaccgataccaggatcttgccatcctatggaactgcctcggtgagttttctccttcattacagaaacggctttttcaaaaatatggtattgataatcctgatatgaataaattgcagtttcatttgatgctcgatgagtttttctaactgtcagaccaagtttactcatatatactttagattgatttaaaacttcatttttaatttaaaaggatctaggtgaagatcctttttgataatctcatgaccaaaatcccttaacgtgagttttcgttccactgagcgtcagaccccgtagaaaagatcaaaggatcttcttgagatcctttttttctgcgcgtaatctgctgcttgcaaacaaaaaaaccaccgctaccagcggtggtttgtttgccggatcaagagctaccaactctttttccgaaggtaactggcttcagcagagcgcagataccaaatactgttcttctagtgtagccgtagttaggccaccacttcaagaactctgtagcaccgcctacatacctcgctctgctaatcctgttaccagtggctgctgccagtggcgataagtcgtgtcttaccgggttggactcaagacgatagttaccggataaggcgcagcggtcgggctgaacggggggttcgtgcacacagcccagcttggagcgaacgacctacaccgaactgagatacctacagcgtgagctatgagaaagcgccacgcttcccgaagggagaaaggcggacaggtatccggtaagcggcagggtcggaacaggagagcgcacgagggagcttccagggggaaacgcctggtatctttatagtcctgtcgggtttcgccacctctgacttgagcgtcgatttttgtgatgctcgtcaggggggcggagcctatggaaaaacgccagcaacgcggcctttttacggttcctggccttttgctggccttttgctcacatgttctttcctgcgttatcccctgattctgtggataacc

SEQ ID NO: 3 - DNA, 23 bp, Homo sapiens
cgccatggcggtctcccgcccgg

SEQ ID NO: 4 - DNA, 23 bp, Homo sapiens
gctgcaccgaccgtgagtttggg

SEQ ID NO: 5 - DNA, 90 bp, Homo sapiens
cctaggtgacacagcaagacgttgtctctggggaaaaaagaaagaaacggaaccacgcggtgtgcagccttctgagtctggcccctttcg

SEQ ID NO: 6 - DNA, 20 bp, Homo sapiens
gctgctgctggaaggacttg

SEQ ID NO: 7 - DNA, 23 bp, Homo sapiens
cgccatggcggtctcccgcccgg

SEQ ID NO: 8 - DNA, 23 bp, Homo sapiens
gctgcaccgaccgtgagtttggg

SEQ ID NO: 9 - DNA, 22 bp, Homo sapiens
ggtaccgttccatcagtccagc

SEQ ID NO: 10 - DNA, 20 bp, Homo sapiens
gagctcgttccatcgctggt

SEQ ID NO: 11 - DNA, 51 bp, Homo sapiens
ttaccagcgatggaacgagctctgaatatgtgaataatcttttcagtcatc

SEQ ID NO: 12 - DNA, 43 bp, Homo sapiens
ttcctcgccttctgcgcctgcaggtcatggaaggtggcgacac

SEQ ID NO: 13 - DNA, 30 bp, Homo sapiens
atgacctgcaggcgcagaaggcgaggaagc

SEQ ID NO: 14 - DNA, 72 bp, Homo sapiens
agacgaattcctaataacttcgtatagcatacattatacgaagttattattacttgtacagctcgtccatgc

SEQ ID NO: 15 - DNA, 72 bp, Homo sapiens
agctgtacaagtaataataacttcgtataatgtatgctatacgaagttattaggaattcgtctgaagaggag

SEQ ID NO: 16 - DNA, 78 bp, Homo sapiens
ccttgctgctggcgcgccataacttcgtataatgtatgctatacgaagttataggcctctagagtcagcttctgatgg

SEQ ID NO: 17 - DNA, 30 bp, Homo sapiens
ttatggcgcgccagcagcaaggcccaggtc

SEQ ID NO: 18 - DNA, 56 bp, Homo sapiens
gctggactgatggaacggtacctggctcacaaaaggaggggcttcactaataactg

SEQ ID NO: 19 - DNA, 20 bp, Homo sapiens
ggtacccagcttttgttccc

SEQ ID NO: 20 - DNA, 25 bp, Homo sapiens
aactgagctccaattcgccctatag

SEQ ID NO: 21 - DNA, 48 bp, Homo sapiens
gggcgaattggagctcagttcctgcaggtgcaggaccaccccaactac

SEQ ID NO: 22 - DNA, 45 bp, Homo sapiens
ttcctcgccttctgcgcctgcagggcacgtcaggatagttgcagt

SEQ ID NO: 23 - DNA, 42 bp, Homo sapiens
aactatcctgacgtgccctgcaggcgcagaaggcgaggaagc

SEQ ID NO: 24 - DNA, 67 bp, Homo sapiens
tcagacgaattcctaataacttcgtatagcatacattatacgaagttattattacttgtacagctcg

SEQ ID NO: 25 - DNA, 65 bp, Homo sapiens
caagtaataataacttcgtataatgtatgctatacgaagttattaggaattcgtctgaagaggag

SEQ ID NO: 26 - DNA, 79 bp, Homo sapiens
ggatcagggacctgggtaccggcgcgccataacttcgtataatgtatgctatacgaagttataggcctctagagtcagc

SEQ ID NO: 27 - DNA, 36 bp, Homo sapiens
ttatggcgcgccggtacccaggtccctgatccgccc

SEQ ID NO: 28 - DNA, 41 bp, Homo sapiens
agggaacaaaagctgggtacccttgccacttcccaaggtgt

SEQ ID NO: 29 - DNA, 22 bp, Homo sapiens
ccaattcgccctatagtgagtc

SEQ ID NO: 30 - DNA, 20 bp, Homo sapiens
ctccagcttttgttcccttt

SEQ ID NO: 31 - DNA, 42 bp, Homo sapiens
actaaagggaacaaaagctggatgtacaacatgatggagacg

SEQ ID NO: 32 - DNA, 32 bp, Homo sapiens
ctcgcccttgctcaccatgtgtgagaggggca

SEQ ID NO: 33 - DNA, 27 bp, Homo sapiens
ctctcacacatggtgagcaagggcgag

SEQ ID NO: 34 - DNA, 30 bp, Homo sapiens
ctctgccctccttgtacagctcgtccatgc

SEQ ID NO: 35 - DNA, 29 bp, Homo sapiens
gctgtacaaggagggcagaggaagtcttc

SEQ ID NO: 36 - DNA, 30 bp, Homo sapiens
tgtccggcccttagccctcccacacataac

SEQ ID NO: 37 - DNA, 28 bp, Homo sapiens
ggagggctaagggccggacagcgaactg

SEQ ID NO: 38 - DNA, 28 bp, Homo sapiens
ggagggctaagggccggacagcgaactg

SEQ ID NO: 39 - DNA, 23 bp, Homo sapiens
gaggggtgtgtagtgcgcggggg

SEQ ID NO: 40 - DNA, 23 bp, Homo sapiens
gcagtaatataccgcggagctgg

SEQ ID NO: 41 - DNA, 23 bp, Homo sapiens
gtgcccggcacggccattaacgg

SEQ ID NO: 42 - DNA, 25 bp, Homo sapiens
caccgtcccaagcagctgaactaca

SEQ ID NO: 43 - DNA, 24 bp, Homo sapiens
caccgtcgcgtgttgcccacgcgt

SEQ ID NO: 44 - DNA, 24 bp, Homo sapiens
caccggcattatgaacctacttcg

SEQ ID NO: 45 - DNA, 6721 bp, Homo sapiens
tggtcctgcaactttatccgcctccatccagtctattaattgttgccgggaagctagagtaagtagttcgccagttaatagtttgcgcaacgttgttgccattgctacaggcatcgtggtgtcacgctcgtcgtttggtatggcttcattcagctccggttcccaacgatcaaggcgagttacatgatcccccatgttgtgcaaaaaagcggttagctccttcggtcctccgatcgttgtcagaagtaagttggccgcagtgttatcactcatggttatggcagcactgcataattctcttactgtcatgccatccgtaagatgcttttctgtgactggtgagtactcaaccaagtcattctgagaatagtgtatgcggcgaccgagttgctcttgcccggcgtcaatacgggataataccgcgccacatagcagaactttaaaagtgctcatcattggaaaacgttcttcggggcgaaaactctcaaggatcttaccgctgttgagatccagttcgatgtaacccactcgtgcacccaactgatcttcagcatcttttactttcaccagcgtttctgggtgagcaaaaacaggaaggcaaaatgccgcaaaaaagggaataagggcgacacggaaatgttgaatactcatactcttcctttttcaatattattgaagcatttatcagggttattgtctcatgagcggatacatatttgaatgtatttagaaaaataaacaaataggggttccgcgcacatttccccgaaaagtgccacctaaattgtaagcgttaatattttgttaaaattcgcgttaaatttttgttaaatcagctcattttttaaccaataggccgaaatcggcaaaatcccttataaatcaaaagaatagaccgagatagggttgagtgttgttccagtttggaacaagagtccactattaaagaacgtggactccaacgtcaaagggcgaaaaaccgtctatcagggcgatggcccactacgtgaaccatcaccctaatcaagttttttggggtcgaggtgccgtaaagcactaaatcggaaccctaaagggagcccccgatttagagcttgacggggaaagccggcgaacgtggcgagaaaggaagggaagaaagcgaaaggagcgggcgctagggcgctggcaagtgtagcggtcacgctgcgcgtaaccaccacacccgccgcgcttaatgcgccgctacagggcgcgtcccattcgccattcaggctgcgcaactgttgggaagggcgatcggtgcgggcctcttcgctattacgccagctggcgaaagggggatgtgctgcaaggcgattaagttgggtaacgccagggttttcccagtcacgacgttgtaaaacgacggccagtgaattaccagcgatggaacgagctctttctcacctggcctccttcagcatttctgtccctcagtccttagcaagcccaggagctgttgagtttggcaggtgccgagtgctgttcctgcctgtgtagctgtggctcagtcctgtgggggccccgctgtggcccgagtgcagtgattcgaggcgctgagtgttccctgactccttctccaggagctgtgttcagactttcgcagctcttggcttggagctcctggagggcttggcattgccgaccaatgtggaggtcgacagtgagagaggaggaatgctagctttcttgaccagtccattaaataagtgggatattggccaggcacggcggctcacgccttaatcccagcactttgggaggctgaggcgggtggatcacgagctcaggagttcaagaccagcctggccaacatggtgaaaccccctctatactaaaaatacaaatattagctgggcgtggtggcaggcgcctgtaatcctagctacttgggaggctgaggcaggagaacagcttgaaaccggaaggtggagtttgcagtgagccaagattgcgccactgcactccaacctgggcaacaagagcaaaactctatctcaaaaaaaaaaaaaaaagtaggatatctgtttctgcttagaaaaatcagaattttctaaatgccaggtgttctgaatacgtaagtatgggagacgactcagcctgtttcatttttatgtaaaatcttcgcgtagccatgtggcactggaccgagatgaaagcaaagacatttctccttaactttgtttctaggaatgttccggagaatcacagcagctgccactaggctgttccgcagtgatggctgtggcggcagtttctacaccctggacagcttgaacttgcgggctcgttccatgatcaccacccacccggccctggtgctgctctggtgtcagatactgctgcttgtcaaccacaccgactaccgctggtgggcagaagtgcagcagaccccgaacctaggtgacacagcaagacgttgtctctggggaaaaaagaaagaaacggaaccacgcggtgtgcagccttctgagtctggcccctttcggtaggttcataatgccccacagcccagggcgccagcccagataacttcgtatagcatacattatacgaagttattaggaattcgtctgaagaggagtttacgtccagccaagcttaggatctcgacctcgaaattctaccgggtaggggaggcgcttttcccaaggcagtctggagcatgcgctttagcagccccgctgggcacttggcgctacacaagtggcctctggcctcgcacacattccacatccaccggtaggcgccaaccggctccgttctttggtggccccttcgcgccaccttctactcctcccctagtcaggaagttcccccccgccccgcagctcgcgtcgtgcaggacgtgacaaatggaagtagcacgtctcactagtctcgtgcagatggacagcaccgctgagcaatggaagcgggtaggcctttggggcagcggccaatagcagctttgctccttcgctttctgggctcagaggctgggaaggggtgggtccgggggcgggctcaggggcgggctcaggggcggggcgggcgcccgaaggtcctccggaggcccggcattctgcacgcttcaaaagcgcacgtctgccgcgctgttctcctcttcctcatctccgggcctttcgacctgcatccatctagatctcgagcagctgaagcttagctagcatgaccgagtacaagcccacggtgcgcctcgccacccgcgacgacgtcccccgggccgtacgcaccctcgccgccgcgttcgccgactaccccgccacgcgccacaccgtcgacccggaccgccacatcgagcgggtcaccgagctgcaagaactcttcctcacgcgcgtcgggctcgacatcggcaaggtgtgggtcgcggacgacggcgccgcggtggcggtctggaccacgccggagagcgtcgaagcgggggcggtgttcgccgagatcggcccgcgcatggccgagttgagcggttcccggctggccgcgcagcaacagatggaaggcctcctggcgccgcaccggcccaaggagcccgcgtggttcctggccaccgtcggcgtctcgcccgaccaccagggcaagggtctgggcagcgccgtcgtgctccccggagtggaggcggccgagcgcgccggggtgcccgccttcctggagacctccgcgccccgcaacctccccttctacgagcggctcggcttcaccgtcaccgccgacgtcgaggtgcccgaaggaccgcgcacctggtgcatgacccgcaagcccggtgcctgaggatcctctgcagaaattgatgatctattaaacaataaagatgtccactaaaatggaagtttttcctgtcatactttgttaagaagggtgagaacagagtacctacattttgaatggaaggattggagctacgggggtgggggtggggtgggattagataaatgcctgctctttactgaaggctctttactattgctttatgataatgtttcatagttggatatcataatttaaacaagcaaaaccaaattaagggccagctcattcctcccactcatgatctatagatctatagatctctcgtgggatcattgtttttctcttgattcccactttgtggttctaagtactgtggtttccaaatgtgtcagtttcatagcctgaagaacgagatcagcagcctctgttccacatacacttcattctcagtattgttttgccaagttctaattccatcagaagctgactctagaggcctataacttcgtatagcatacattatacgaagttatcaccctgtcctgagactcccagtaacctgagctttggccaccgttaaagcattttcattttccattttttgtgagggcttgtgaaatttctgctgcatattaatattcctttcatggacagcatattattgggacaaacatgcggtccagctaaaggcattcaaaatagcagttgctttctaaatgcgattttctttggcaggttctttgacaccattgcatcttgtgggatatgcttgtcatgctctgtggctcctactaagttctagtccttaaattggttccatagccagacatgttgcaatgtcttaacctcattataaagtaaatgtggttctggttatccttagataatgaagtaacagtgtagcaaatttcaaaacctcttggaaatgttattttaccattcaaaaaggcttactaaggttctcgttatgggtggccctctttttgcaaaaggttttcaggcttaagctccatttctaggtgctccaacactccattatttgtatatgtatggaaataaaagctgtgaccacccccaaccctggcccccgcccagctgaatcctcagcacagtatttctggaaggctcaagatcccacgctggggaaaagaagttctggagacaaaagagggcaggtgctgccgtgcctctctgctcagtatggatactggaccttgtgctgccagggctcccagtagggccagttcatggcactcagctggaaagtccactgttgggaggcattcttaaccatccactctgtgccgtatgtagtggggtctggtcattctgttggaggagacagaccagtgacgacatttgaaatgcttggtggatgtcttaggcctgttacgatgactgagcactgtgggggcaggagacagaaagtcagtgtctcctagttctgtgctgctttaacgtgcatagaaatcagctgcggattcagcagatcactccttttctgacagatgggcctgcttactctgatgttatttgtgagccaggtaccgttccatcagtccagcttggcgtaatcatggtcatagctgtttcctgtgtgaaattgttatccgctcacaattccacacaacatacgagccggaagcataaagtgtaaagcctggggtgcctaatgagtgagctaactcacattaattgcgttgcgctcactgcccgctttccagtcgggaaacctgtcgtgccagctgcattaatgaatcggccaacgcgcggggagaggcggtttgcgtattgggcgctcttccgcttcctcgctcactgactcgctgcgctcggtcgttcggctgcggcgagcggtatcagctcactcaaaggcggtaatacggttatccacagaatcaggggataacgcaggaaagaacatgtgagcaaaaggccagcaaaaggccaggaaccgtaaaaaggccgcgttgctggcgtttttccataggctccgcccccctgacgagcatcacaaaaatcgacgctcaagtcagaggtggcgaaacccgacaggactataaagataccaggcgtttccccctggaagctccctcgtgcgctctcctgttccgaccctgccgcttaccggatacctgtccgcctttctcccttcgggaagcgtggcgctttctcatagctcacgctgtaggtatctcagttcggtgtaggtcgttcgctccaagctgggctgtgtgcacgaaccccccgttcagcccgaccgctgcgccttatccggtaactatcgtcttgagtccaacccggtaagacacgacttatcgccactggcagcagccactggtaacaggattagcagagcgaggtatgtaggcggtgctacagagttcttgaagtggtggcctaactacggctacactagaaggacagtatttggtatctgcgctctgctgaagccagttaccttcggaaaaagagttggtagctcttgatccggcaaacaaaccaccgctggtagcggtggtttttttgtttgcaagcagcagattacgcgcagaaaaaaaggatctcaagaagatcctttgatcttttctacggggtctgacgctcagtggaacgaaaactcacgttaagggattttggtcatgagattatcaaaaaggatcttcacctagatccttttaaattaaaaatgaagttttaaatcaatctaaagtatatatgagtaaacttggtctgacagttaccaatgcttaatcagtgaggcacctatctcagcgatctgtctatttcgttcatccatagttgcctgactccccgtcgtgtagataactacgatacgggagggcttaccatctggccccagtgctgcaatgataccgcgagacccacgctcaccggctccagatttatcagcaataaaccagccagccggaagggccgagcgcagaag

SEQ ID NO: 46 - DNA, 18 bp, Homo sapiens
cgtgaattgctgccctct

SEQ ID NO: 47 - DNA, 20 bp, Homo sapiens
cagaaacccctagcttccaa

SEQ ID NO: 48 - DNA, 19 bp, Homo sapiens
cccagagccccattcattg

SEQ ID NO: 49 - DNA, 20 bp, Homo sapiens
aggacaagggaagacccaag

SEQ ID NO: 50 - DNA, 93 bp, Mus musculus
cagagggtgcctggtgaaatgccttttgtaccatctgttgtcagatacaaacagtaccatcattccaggaagttccctcttgtccctttatca

SEQ ID NO: 51 - DNA, 99 bp, Unknown
  Description of Unknown: Marmoset oligonucleotide
tccctggtgacagagcaagaccttgtctctggggaaaaaaaattaagaaagaaatggaagcatgcagtgtgcagccttttgagtctgccctctcggtct

SEQ ID NO: 52 - DNA, 98 bp, Macaca sp.
accctaggtgacacagcaagaccttgtctttgggaaaaaaattaagaaagagatggaaccacacagtgtgcagccttttgagtctggccccttgcact

SEQ ID NO: 53 - DNA, 88 bp, Pongo sp.
agcctgggtgacacagcaagaccttgtctctgggagaaagaaacggaaccacgcagtgtgcagccttttgagtctggcccctttcggt

SEQ ID NO: 54 - DNA, 94 bp, Pan troglodytes
agcctaggtgacacagcaagacattgtctctggggaaaaaagaaagaaacggaaccacgcagtgtgcagccttctgagtctggcccctttcggt

SEQ ID NO: 55 - DNA, 94 bp, Gorilla sp.
agcctaggtgacacagcaagacgttgtctctggggaaaaaagaaagaaacggaaccacgcagtgtgcagccttctgagtctggcccctttcggt

SEQ ID NO: 56 - DNA, 94 bp, Homo sapiens
agcctaggtgacacagcaagacgttgtctctggggaaaaaagaaagaaacggaaccacgcggtgtgcagccttctgagtctggcccctttcggt

SEQ ID NO: 57 - DNA, 19 bp, Artificial Sequence
  Description of Artificial Sequence: Synthetic primer
ccaagatggacggccgctc

SEQ ID NO: 58 - DNA, 20 bp, Artificial Sequence
  Description of Artificial Sequence: Synthetic primer
aggacaagggaagacccaag

SEQ ID NO: 59 - DNA, 20 bp, Artificial Sequence
  Description of Artificial Sequence: Synthetic primer
ctccagcttttgttcccttt

SEQ ID NO: 60 - DNA, 22 bp, Artificial Sequence
  Description of Artificial Sequence: Synthetic primer
ccaattcgccctatagtgagtc

SEQ ID NO: 61 - DNA, 39 bp, Artificial Sequence
  Description of Artificial Sequence: Synthetic primer
aaagggaacaaaagctggaggggtcacacttggggtcct

SEQ ID NO: 62 - DNA, 29 bp, Artificial Sequence
  Description of Artificial Sequence: Synthetic primer
tctagggttaaaagcagaacctgagcggc

SEQ ID NO: 63 - DNA, 34 bp, Artificial Sequence
  Description of Artificial Sequence: Synthetic primer
aggttctgcttttaaccctagaaagatagtctgc

SEQ ID NO: 64 - DNA, 36 bp, Artificial Sequence
  Description of Artificial Sequence: Synthetic primer
gggccgcaggttaaccctagaaagataatcatattg

SEQ ID NO: 65 - DNA, 30 bp, Artificial Sequence
  Description of Artificial Sequence: Synthetic primer
tttctagggttaacctgcggcccagagccc

SEQ ID NO: 66 - DNA, 42 bp, Artificial Sequence
  Description of Artificial Sequence: Synthetic primer
gactcactatagggcgaattggcctccccatcagcaacgtgt

SEQ ID NO: 67 - DNA, 22 bp, Artificial Sequence
  Description of Artificial Sequence: Synthetic oligonucleotide
ggtaaaagcagaacctgagcgg

SEQ ID NO: 68 - DNA, 23 bp, Artificial Sequence
  Description of Artificial Sequence: Synthetic oligonucleotide
gctgcaccgaccgtgagtttggg

SEQ ID NO: 69 - DNA, 8759 bp, Artificial Sequence
  Description of Artificial Sequence: Synthetic polynucleotide
gtggcacttttcggggaaatgtgcgcggaacccctatttgtttatttttctaaatacattcaaatatgtatccgctcatgagacaataaccctgataaatgcttcaataatattgaaaaaggaagagtatgagtattcaacatttccgtgtcgcccttattcccttttttgcggcattttgccttcctgtttttgctcacccagaaacgctggtgaaagtaaaagatgctgaagatcagttgggtgcacgagtgggttacatcgaactggatctcaacagcggtaagatccttgagagttttcgccccgaagaacgttttccaatgatgagcacttttaaagttctgctatgtggcgcggtattatcccgtattgacgccgggcaagagcaactcggtcgccgcatacactattctcagaatgacttggttgagtactcaccagtcacagaaaagcatcttacggatggcatgacagtaagagaattatgcagtgctgccataaccatgagtgataacactgcggccaacttacttctgacaacgatcggaggaccgaaggagctaaccgcttttttgcacaacatgggggatcatgtaactcgccttgatcgttgggaaccggagctgaatgaagccataccaaacgacgagcgtgacaccacgatgcctgtagcaatggcaacaacgttgcgcaaactattaactggcgaactacttactctagcttcccggcaacaattaatagactggatggaggcggataaagttgcaggaccacttctgcgctcggcccttccggctggctggtttattgctgataaatctggagccggtgagcgtgggtctcgcggtatcattgcagcactggggccagatggtaagccctcccgtatcgtagttatctacacgacggggagtcaggcaactatggatgaacgaaatagacagatcgctgagataggtgcctcactgattaagcattggtaactgtcagaccaagtttactcatatatactttagattgatttaaaacttcatttttaatttaaaaggatctaggtgaagatcctttttgataatctcatgaccaaaatcccttaacgtgagttttcgttccactgagcgtcagaccccgtagaaaagatcaaaggatcttcttgagatcctttttttctgcgcgtaatctgctgcttgcaaacaaaaaaaccaccgctaccagcggtggtttgtttgccggatcaagagctaccaactctttttccgaaggtaactggcttcagcagagcgcagataccaaatactgtccttctagtgtagccgtagttaggccaccacttcaagaactctgtagcaccgcctacatacctcgctctgctaatcctgttaccagtggctgctgccagtggcgataagtcgtgtcttaccgggttggactcaagacgatagttaccggataaggcgcagcggtcgggctgaacggggggttcgtgcacacagcccagcttggagcgaacgacctacaccgaactgagatacctacagcgtgagctatgagaaagcgccacgcttcccgaagggagaaaggcggacaggtatccggtaagcggcagggtcggaacaggagagcgcacgagggagcttccagggggaaacgcctggtatctttatagtcctgtcgggtttcgccacctctgacttgagcgtcgatttttgtgatgctcgtcaggggggcggagcctatggaaaaacgccagcaacgcggcctttttacggttcctggccttttgctggccttttgctcacatgttctttcctgcgttatcccctgattctgtggataaccgtattaccgcctttgagtgagctgataccgctcgccgcagccgaacgaccgagcgcagcgagtcagtgagcgaggaagcggaagagcgcccaatacgcaaaccgcctctccccgcgcgttggccgattcattaatgcagctggcacgacaggtttcccgactggaaagcgggcagtgagcgcaacgcaattaatgtgagttagctcactcattaggcaccccaggctttacactttatgcttccggctcgtatgttgtgtggaattgtgagcggataacaatttcacacaggaaacagctatgaccatgattacgccaagcgcgcaattaaccctcactaaagggaacaaaagctggagctccaccgcggggcgcgccgcagctagattaaccctagaaagatagtctgcgtaaaattgacgcatgcattcttgaaatattgctctctctttctaaatagcgcgaatccgtcgctgtgcatttaggacatctcagtcgccgcttggagctcccgtgaggcgtgcttgtcaatgcggtaagtgtcactgattttgaactataacaaccgcgtgagtcaaaatgacgcatgattatcttttacgtgacttttaagatttaactcatacgataattatattgttatttcgtgttctacttacgtgataacttattatatatatattttcttgttatagatgggaattcagacatgataagatacattgatgagtttggacaaaccacaactagaatgcagtgaaaaaaatgctttatttgtgaaatttgtgatgctattgctttatttgtaaccattataagctgcaataaacaagtttcgaggtcgagtgtcagtcctgctcctcggccacgaagtgcttagccctcccacacataaccagagggcagcaattcacgaatcccaactgccgtcggctgtccatcactgtccttcactatggctttgatcccaggatgcagatcgagaagcacctgtcggcaccgtccgcaggggctcaagatgcccctgttctcatttccgatcgcgacgatacaagtcaggttgccagctgccgcagcagcagcagtgcccagcaccacgagttctgcacaaggtcccccagtaaaatgatatacattgacaccagtgaagatgcggccgtcgctagagagagctgcgctggcgacgctgtagtcttcagagatggggatgctgttgattgtagccgttgctctttcaatgagggtggattcttcttgagacaaaggcttggccatggtttagttcctcaccttgtcgtattatactatgccgatatactatgccgatgattaattgtcaacacggtccggtctaacaaaaaagccaaaaacggccagaatttagcggacaatttactagtctaacactgaaaattacatattgacccaaatgattacatttcaaaaggtgcctaaaaaacttcacaaaacacactcgccaaccccgagcgcatagttcaaaaccggagcttcagctacttaagaagataggtacataaaaccgaccaaagaaactgacgcctcacttatccctcccctcaccagaggtccggcgcctgtcgattcaggagagcctaccctaggcccgaaccctgcgtcctgcgacggagaaaagcctaccgcacacctaccggcaggtggccccaccctgcattataagccaacagaacgggtgacgtcacgacacgacgagggcgcgcgctcccaaaggtacgggtgcactgcccaacggcaccgccataactgccgcccccgcaacagacgacaaaccgagttctccagtcagtgacaaacttcacgtcagggtccccagatggtgccccagcccatctcacccgaataagagctttcccgcattagcgaaggcctcaagaccttgggttcttgccgcccaccatgccccccaccttgtttcaacgacctcacagcccgcctcacaagcgtcttccattcaagactcgggaacagccgccattttgctgcgctccccccaacccccagttcagggcaaccttgctcgcggacccagactacagcccttggcggtctctccacacgcttccgtcccaccgagcggcccggcggccacgaaagccccggccagcccagcagcccgctactcaccaagtgacgatcacagcgatccacaaacaagaaccgcgacccaaatcccggctgcgacggaactagctgtgccacacccggcgcgtccttatataatcatcggcgttcaccgccccacggagatccctccgcagaatcgccgagaagggactacttttcctcgcctgttccgctctctggaaagaaaaccagtgccctagagtcacccaagtcccgtcctaaaatgtccttctgctgatactggggttctaaggccgagtcttatgagcagcgggccgctgtcctgagcgtccgggcggaaggatcaggacgctcgtgcgcccttcgtctgacgtggcagcgctcgccgtgaggagggggcgcccgcggggggcgccaaaacccggcgcggaggccagatctcccgatctcgagcgacattgattattgactagttattaatagtaatcaattacggggtcattagttcatagcccatatatggagttccgcgttacataacttacggtaaatggcccgcctggctgaccgcccaacgacccccgcccattgacgtcaataatgacgtatgttcccatagtaacgccaatagggactttccattgacgtcaatgggtggagtatttacggtaaactgcccacttggcagtacatcaagtgtatcatatgccaagtacgccccctattgacgtcaatgacggtaaatggcccgcctggcattatgcccagtacatgaccttatgggactttcctacttggcagtacatctacgtattagtcatcgctattaccatggtcgaggtgagccccacgttctgcttcactctccccatctcccccccctccccacccccaattttgtatttatttattttttaattattttgtgcagcgatgggggcggggggggggggggggcgcgcgccaggcggggcggggcggggcgaggggcggggcggggcgaggcggagaggtgcggcggcagccaatcagagcggcgcgctccgaaagtttccttttatggcgaggcggcggcggcggcggccctataaaaagcgaagcgcgcggcgggcgggagtcgctgcgcgctgccttcgccccgtgccccgctccgccgccgcctcgcgccgcccgccccggctctgactgaccgcgttactcccacaggtgagcgggcgggacggcccttctcctccgggctgtaattagcgcttggtttaatgacggcttgtttcttttctgtggctgcgtgaaagccttgaggggctccgggagggccctttgtgcggggggagcggctcggggggtgcgtgcgtgtgtgtgtgcgtggggagcgccgcgtgcggctccgcgctgcccggcggctgtgagcgctgcgggcgcggcgcggggctttgtgcgctccgcagtgtgcgcgaggggagcgcggccgggggcggtgccccgcggtgcggggggggctgcgaggggaacaaaggctgcgtgcggggtgtgtgcgtgggggggtgagcagggggtgtgggcgcgtcggtcgggctgcaaccccccctgcacccccctccccgagttgctgagcacggcccggcttcgggtgcggggctccgtacggggcgtggcgcggggctcgccgtgccgggcggggggtggcggcaggtgggggtgccgggcggggcggggccgcctcgggccggggagggctcgggggaggggcgcggcggcccccggagcgccggcggctgtcgaggcgcggcgagccgcagccattgccttttatggtaatcgtgcgagagggcgcagggacttcctttgtcccaaatctgtgcggagccgaaatctgggaggcgccgccgcaccccctctagcgggcgcggggcgaagcggtgcggcgccggcaggaaggaaatgggcggggagggccttcgtgcgtcgccgcgccgccgtccccttctccctctccagcctcggggctgtccgcggggggacggctgccttcgggggggacggggcagggcggggttcggcttctggcgtgtgaccggcggctctagagcctctgctaaccatgttcatgccttcttctttttcctacagctcctgggcaacgtgctggttattgtgctgtctcatcattttggcaaagaattaaatttaattaatctcgacggtatcggttaacgaatccaagggcgaattccagcacactggcggccgttactagtggatccaagcttgccaccatggcggaaggatccgtcgccaggcagcctgacctcttgacctgcgacgatgagccgatccatatccccggtgccatccaaccgcatggactgctgctcgccctcgccgccgacatgacgatcgttgccggcagcgacaaccttcccgaactcaccggactggcgatcggcgccctgatcggccgctctgcggccgatgtcttcgactcggagacgcacaaccgtctgacgatcgccttggccgagcccggggcggccgtcggagcaccgatcactgtcggcttcacgatgcgaaaggacgcaggcttcatcggctcctggcatcgccatgatcagctcatcttcctcgagctcgagcctccccagcgggacgtcgccgagccgcaggcgttcttccgccgcaccaacagcgccatccgccgcctgcaggccgccgaaaccttggaaagcgcctgcgccgccgcggcgcaagaggtgcggaagattaccggcttcgatcgggtgatgatctatcgcttcgcctccgacttcagcggcgaagtgatcgcagaggatcggtgcgccgaggtcgagtcaaaactaggcctgcactatcctgcctcaaccgtgccggcgcaggcccgtcggctctataccatcaacccggtacggatcattcccgatatcaattatcggccggtgccggtcaccccagacctcaatccggtcaccgggcggccgattgatcttagcttcgccatcctgcgcagcgtctcgcccgtccatctggagttcatgcgcaacataggcatgcacggcacgatgtcgatctcgattttgcgcggcgagcgactgtggggattgatcgtttgccatcaccgaacgccgtactacgtcgatctcgatggccgccaagcctgcgagctagtcgcccaggttctggcctggcagatcggcgtgatggaagagggaggtagtggatcaatgccagagccagcgaagtctgctcccgccccgaaaaagggctccaagaaggcggtgactaaggcgcagaagaaaggcggcaagaagcgcaagcgcagccgcaaggagagctattccatctatgtgtacaaggttctgaagcaggtccaccctgacaccggcatttcgtccaaggccatgggcatcatgaattcgtttgtgaacgacattttcgagcgcatcgcaggtgaggcttcccgcctggcgcattacaacaagcgctcgaccatcacctccagggagatccagacggccgtgcgcctgctgctgcctggggagttggccaagcacgccgtgtccgagggtactaaggccatcaccaagtacaccagcgctaagtgagcggccgcgactctagatcataatcagccataccacatttgtagaggttttacttgctttaaaaaacctcccacacctccccctgaacctgaaacataaaatgaatgcaattgttgttgttaacttgtttattgcagcttataatggttacaaataaagcaatagcatcacaaatttcacaaataaagcatttttttcactgcattctagttgtggtttgtccaaactcatcaatgtatcttaaggaattcgataaaagttttgttactttatagaagaaattttgagtttttgtttttttttaataaataaataaacataaataaattgtttgttgaatttattattagtatgtaagtgtaaatataataaaacttaatatctattcaaattaataaataaacctcgatatacagaccgataaaacacatgcgtcaattttacgcatgattatctttaacgtacgtcacaatatgattatctttctagggttaatctagctgcggcgcgccggtacccaattcgccctatagtgagtcgtattacgcgcgctcactggccgtcgttttacaacgtcgtgactgggaaaaccctggcgttacccaacttaatcgccttgcagcacatccccctttcgccagctggcgtaatagcgaagaggcccgcaccgatcgcccttcccaacagttgcgcagcctgaatggcgaatgggacgcgccctgtagcggcgcattaagcgcggcgggtgtggtggttacgcgcagcgtgaccgctacacttgccagcgccctagcgcccgctcctttcgctttcttcccttcctttctcgccacgttcgccggctttccccgtcaagctctaaatcgggggctccctttagggttccgatttagtgctttacggcacctcgaccccaaaaaacttgattagggtgatggttcacgtagtgggccatcgccctgatagacggtttttcgccctttgacgttggagtccacgttctttaatagtggactcttgttccaaactggaacaacactcaaccctatctcggtctattcttttgatttataagggattttgccgatttcggcctattggttaaaaaatgagctgatttaacaaaaatttaacgcgaattttaacaaaatattaacgcttacaatttag

SEQ ID NO: 70 - DNA, 6 bp, Artificial Sequence
  Description of Artificial Sequence: Synthetic oligonucleotide
caacag